European Patent Application EP 4 570 248 A1, published June 18, 2025. Title: SIROLIMUS-CONTAINING TOPICAL DRUG FOR TREATING SKIN HARDENING IN SYSTEMIC SCLERODERMA. Applicant: NATIONAL UNIVERSITY CORPORATION GUNMA UNIVERSITY. Application EP 23852589.3, filed August 9, 2023. The sequence listing filed with the application follows.

SEQUENCE LISTING (4 sequences)

SEQ ID NO: 1 - DNA, 21 bp, synthetic construct
  source 1..21: mol_type = other DNA
gcctcttctcattcctgcttg

SEQ ID NO: 2 - DNA, 20 bp, synthetic construct
  source 1..20: mol_type = other DNA
ctgatgagagggaggccatt

SEQ ID NO: 3 - DNA, 20 bp, synthetic construct
  source 1..20: mol_type = other DNA
tacggcagtggctgaaccaa

SEQ ID NO: 4 - DNA, 21 bp, synthetic construct
  source 1..21: mol_type = other DNA
cggttcatgtcatggatggtg